European Patent Application EP 4 656 653 A2, published December 3, 2025. Title: Tethered interleukin-15 and interleukin-21. Applicant: The United States of America, as represented by The Secretary, Department of Health and Human Services. Application EP. The sequence listing filed with the application follows.

SEQUENCE LISTING (44 sequences)

SEQ ID NO: 1 - protein, 18 aa, Homo sapiens
MDWTWILFLVAAATRVHS

SEQ ID NO: 2 - protein, 133 aa, Homo sapiens [sequence omitted]

SEQ ID NO: 3 - protein, 114 aa, Homo sapiens
NWVNVISDLKKIEDLIQSMHIDATLYTESDVHPSCKVTAMKCFLLELQVISLESGDASIHDTVENLIILANNSLSSNGNVTESGCKECEELEEKNIKEFLQSFVHIVQMFINTS

SEQ ID NO: 4 - protein, 21 aa, Homo sapiens
IYIWAPLAGTCGVLLLSLVIT

SEQ ID NO: 5 - protein, 46 aa, Homo sapiens
LLPSWAITLISVNGIFVICCLTYCFAPRCRERRRNERLRRESVRPV

SEQ ID NO: 6 - protein, 9 aa, porcine teschovirus-1 2A
  SITE 5: note = MISC_FEATURE - X is any naturally occurring amino acid residue.
GDVEXNPGP

SEQ ID NO: 7 - protein, 22 aa, porcine teschovirus-1 2A
GSGATNFSLLKQAGDVEENPGP

SEQ ID NO: 8 - protein, 23 aa, equine rhinitis A virus 2a
GSGQCTNYALLKLAGDVESNPGP

SEQ ID NO: 9 - protein, 21 aa, thosea asigna virus 2A
GSGEGRGSLLTCGDVEENPGP

SEQ ID NO: 10 - skipped

SEQ ID NO: 11 - protein, 27 aa, synthetic construct
  REGION 1..27: note = synthetic
RAKRSGSGATNFSLLKQAGDVEENPGP

SEQ ID NO: 12 - protein, 27 aa, synthetic construct
  REGION 1..27: note = synthetic
SGGGGSGGGGSGGGGSGGGGSGGGSLQ

SEQ ID NO: 13 - protein, 18 aa, synthetic construct
  REGION 1..18: note = synthetic
GSTSGSGKPGSGEGSTKG

SEQ ID NO: 14 - protein, 45 aa, synthetic construct
  REGION 1..45: note = synthetic
GGGGSGGGGSGGGGSGGGGSGGGGSGGGGSGGGGSGGGGSGGGGS

SEQ ID NO: 15 - protein, 46 aa, synthetic construct
  REGION 1..46: note = synthetic
AEAAAKEAAAKEAAAKEAAAKALEAEAAAKEAAAKEAAAKEAAAKA

SEQ ID NO: 16 - protein, 48 aa, synthetic construct
  REGION 1..48: note = synthetic
SGGGGSGGGGSGGGGSGGGGSGGGGSGGGGSGGGGSGGGGSGGGGSLQ

SEQ ID NO: 17 - protein, 61 aa, synthetic construct
  REGION 1..61: note = synthetic
AGGGSGGGGSGGGGSGGGGSGGGGSGGGGSGGGGSGGGGSGGGGSGGGSGGGGSGGGGSAS

SEQ ID NO: 18 - protein, 237 aa, synthetic construct
  REGION 1..237: note = synthetic
ITCPPPMSVEHADIWVKSYSLYSRERYICNSGFKRKAGTSSLTECVLNKATNVAHWTTPSLKCIRDPALVHQRPAPPSTVTTAGVTPQPESLSPSGKEPAASSPSSNNTAATTAAIVPGSQLMPSKSPSTGTTEISSHESSHGTPSQTTAKNWELTASASHQPPGVYPQGHSDTTVAISTSTVLLCGLSAVSLLACYLKSRQTPPLASVEMEAMEALPVTWGTSSRDEDLENCSHHL

SEQ ID NO: 19 - protein, 180 aa, synthetic construct
  REGION 1..180: note = synthetic
MDWTWILFLVAAATRVHSNWVNVISDLKKIEDLIQSMHIDATLYTESDVHPSCKVTAMKCFLLELQVISLESGDASIHDTVENLIILANNSLSSNGNVTESGCKECEELEEKNIKEFLQSFVHIVQMFINTSSGGGGSGGGGSGGGGSGGGGSGGGSLQIYIWAPLAGTCGVLLLSLVIT

SEQ ID NO: 20 - protein, 171 aa, synthetic construct
  REGION 1..171: note = synthetic
MDWTWILFLVAAATRVHSNWVNVISDLKKIEDLIQSMHIDATLYTESDVHPSCKVTAMKCFLLELQVISLESGDASIHDTVENLIILANNSLSSNGNVTESGCKECEELEEKNIKEFLQSFVHIVQMFINTSGSTSGSGKPGSGEGSTKGIYIWAPLAGTCGVLLLSLVIT

SEQ ID NO: 21 - protein, 396 aa, synthetic construct
  REGION 1..396: note = synthetic
MDWTWILFLVAAATRVHSNWVNVISDLKKIEDLIQSMHIDATLYTESDVHPSCKVTAMKCFLLELQVISLESGDASIHDTVENLIILANNSLSSNGNVTESGCKECEELEEKNIKEFLQSFVHIVQMFINTSSGGGGSGGGGSGGGGSGGGGSGGGSLQITCPPPMSVEHADIWVKSYSLYSRERYICNSGFKRKAGTSSLTECVLNKATNVAHWTTPSLKCIRDPALVHQRPAPPSTVTTAGVTPQPESLSPSGKEPAASSPSSNNTAATTAAIVPGSQLMPSKSPSTGTTEISSHESSHGTPSQTTAKNWELTASASHQPPGVYPQGHSDTTVAISTSTVLLCGLSAVSLLACYLKSRQTPPLASVEMEAMEALPVTWGTSSRDEDLENCSHHL

SEQ ID NO: 22 - protein, 198 aa, synthetic construct
  REGION 1..198: note = synthetic
MDWTWILFLVAAATRVHSNWVNVISDLKKIEDLIQSMHIDATLYTESDVHPSCKVTAMKCFLLELQVISLESGDASIHDTVENLIILANNSLSSNGNVTESGCKECEELEEKNIKEFLQSFVHIVQMFINTSGGGGSGGGGSGGGGSGGGGSGGGGSGGGGSGGGGSGGGGSGGGGSIYIWAPLAGTCGVLLLSLVIT

SEQ ID NO: 23 - protein, 132 aa, synthetic construct
  REGION 1..132: note = synthetic
MDWTWILFLVAAATRVHSNWVNVISDLKKIEDLIQSMHIDATLYTESDVHPSCKVTAMKCFLLELQVISLESGDASIHDTVENLIILANNSLSSNGNVTESGCKECEELEEKNIKEFLQSFVHIVQMFINTS

SEQ ID NO: 24 - protein, 199 aa, synthetic construct
  REGION 1..199: note = synthetic
MDWTWILFLVAAATRVHSQGQDRHMIRMRQLIDIVDQLKNYVNDLVPEFLPAPEDVETNCEWSAFSCFQKAQLKSANTGNNERIINVSIKKLKRKPPSTNAGRRQKHRLTCPSCDSYEKKPPKEFLERFKSLLQKMIHQHLSSRTHGSEDSSGGGGSGGGGSGGGGSGGGGSGGGSLQIYIWAPLAGTCGVLLLSLVIT

SEQ ID NO: 25 - protein, 190 aa, synthetic construct
  REGION 1..190: note = synthetic
MDWTWILFLVAAATRVHSQGQDRHMIRMRQLIDIVDQLKNYVNDLVPEFLPAPEDVETNCEWSAFSCFQKAQLKSANTGNNERIINVSIKKLKRKPPSTNAGRRQKHRLTCPSCDSYEKKPPKEFLERFKSLLQKMIHQHLSSRTHGSEDSGSTSGSGKPGSGEGSTKGIYIWAPLAGTCGVLLLSLVIT

SEQ ID NO: 26 - protein, 217 aa, synthetic construct
  REGION 1..217: note = synthetic
MDWTWILFLVAAATRVHSQGQDRHMIRMRQLIDIVDQLKNYVNDLVPEFLPAPEDVETNCEWSAFSCFQKAQLKSANTGNNERIINVSIKKLKRKPPSTNAGRRQKHRLTCPSCDSYEKKPPKEFLERFKSLLQKMIHQHLSSRTHGSEDSGGGGSGGGGSGGGGSGGGGSGGGGSGGGGSGGGGSGGGGSGGGGSIYIWAPLAGTCGVLLLSLVIT

SEQ ID NO: 27 - protein, 218 aa, synthetic construct
  REGION 1..218: note = synthetic
MDWTWILFLVAAATRVHSQGQDRHMIRMRQLIDIVDQLKNYVNDLVPEFLPAPEDVETNCEWSAFSCFQKAQLKSANTGNNERIINVSIKKLKRKPPSTNAGRRQKHRLTCPSCDSYEKKPPKEFLERFKSLLQKMIHQHLSSRTHGSEDSAEAAAKEAAAKEAAAKEAAAKALEAEAAAKEAAAKEAAAKEAAAKAIYIWAPLAGTCGVLLLSLVIT

SEQ ID NO: 28 - protein, 220 aa, synthetic construct
  REGION 1..220: note = synthetic
MDWTWILFLVAAATRVHSQGQDRHMIRMRQLIDIVDQLKNYVNDLVPEFLPAPEDVETNCEWSAFSCFQKAQLKSANTGNNERIINVSIKKLKRKPPSTNAGRRQKHRLTCPSCDSYEKKPPKEFLERFKSLLQKMIHQHLSSRTHGSEDSSGGGGSGGGGSGGGGSGGGGSGGGGSGGGGSGGGGSGGGGSGGGGSLQIYIWAPLAGTCGVLLLSLVIT

SEQ ID NO: 29 - protein, 233 aa, synthetic construct
  REGION 1..233: note = synthetic
MDWTWILFLVAAATRVHSQGQDRHMIRMRQLIDIVDQLKNYVNDLVPEFLPAPEDVETNCEWSAFSCFQKAQLKSANTGNNERIINVSIKKLKRKPPSTNAGRRQKHRLTCPSCDSYEKKPPKEFLERFKSLLQKMIHQHLSSRTHGSEDSAGGGSGGGGSGGGGSGGGGSGGGGSGGGGSGGGGSGGGGSGGGGSGGGSGGGGSGGGGSASIYIWAPLAGTCGVLLLSLVIT

SEQ ID NO: 30 - protein, 245 aa, synthetic construct
  REGION 1..245: note = synthetic
MDWTWILFLVAAATRVHSQGQDRHMIRMRQLIDIVDQLKNYVNDLVPEFLPAPEDVETNCEWSAFSCFQKAQLKSANTGNNERIINVSIKKLKRKPPSTNAGRRQKHRLTCPSCDSYEKKPPKEFLERFKSLLQKMIHQHLSSRTHGSEDSSGGGGSGGGGSGGGGSGGGGSGGGGSGGGGSGGGGSGGGGSGGGGSLQLLPSWAITLISVNGIFVICCLTYCFAPRCRERRRNERLRRESVRPV

SEQ ID NO: 31 - protein, 205 aa, synthetic construct
  REGION 1..205: note = synthetic
MDWTWILFLVAAATRVHSNWVNVISDLKKIEDLIQSMHIDATLYTESDVHPSCKVTAMKCFLLELQVISLESGDASIHDTVENLIILANNSLSSNGNVTESGCKECEELEEKNIKEFLQSFVHIVQMFINTSSGGGGSGGGGSGGGGSGGGGSGGGSLQLLPSWAITLISVNGIFVICCLTYCFAPRCRERRRNERLRRESVRPV

SEQ ID NO: 32 - protein, 447 aa, synthetic construct
  REGION 1..447: note = synthetic
MDWTWILFLVAAATRVHSQGQDRHMIRMRQLIDIVDQLKNYVNDLVPEFLPAPEDVETNCEWSAFSCFQKAQLKSANTGNNERIINVSIKKLKRKPPSTNAGRRQKHRLTCPSCDSYEKKPPKEFLERFKSLLQKMIHQHLSSRTHGSEDSSGGGGSGGGGSGGGGSGGGGSGGGGSGGGGSGGGGSGGGGSGGGGSLQIYIWAPLAGTCGVLLLSLVITGSGATNFSLLKQAGDVEENPGPMDWTWILFLVAAATRVHSNWVNVISDLKKIEDLIQSMHIDATLYTESDVHPSCKVTAMKCFLLELQVISLESGDASIHDTVENLIILANNSLSSNGNVTESGCKECEELEEKNIKEFLQSFVHIVQMFINTSSGGGGSGGGGSGGGGSGGGGSGGGSLQLLPSWAITLISVNGIFVICCLTYCFAPRCRERRRNERLRRESVRPV

SEQ ID NO: 33 - protein, 448 aa, synthetic construct
  REGION 1..448: note = synthetic
MDWTWILFLVAAATRVHSQGQDRHMIRMRQLIDIVDQLKNYVNDLVPEFLPAPEDVETNCEWSAFSCFQKAQLKSANTGNNERIINVSIKKLKRKPPSTNAGRRQKHRLTCPSCDSYEKKPPKEFLERFKSLLQKMIHQHLSSRTHGSEDSSGGGGSGGGGSGGGGSGGGGSGGGGSGGGGSGGGGSGGGGSGGGGSLQIYIWAPLAGTCGVLLLSLVITGSGQCTNYALLKLAGDVESNPGPMDWTWILFLVAAATRVHSNWVNVISDLKKIEDLIQSMHIDATLYTESDVHPSCKVTAMKCFLLELQVISLESGDASIHDTVENLIILANNSLSSNGNVTESGCKECEELEEKNIKEFLQSFVHIVQMFINTSSGGGGSGGGGSGGGGSGGGGSGGGSLQLLPSWAITLISVNGIFVICCLTYCFAPRCRERRRNERLRRESVRPV

SEQ ID NO: 34 - protein, 446 aa, synthetic construct
  REGION 1..446: note = synthetic
MDWTWILFLVAAATRVHSQGQDRHMIRMRQLIDIVDQLKNYVNDLVPEFLPAPEDVETNCEWSAFSCFQKAQLKSANTGNNERIINVSIKKLKRKPPSTNAGRRQKHRLTCPSCDSYEKKPPKEFLERFKSLLQKMIHQHLSSRTHGSEDSSGGGGSGGGGSGGGGSGGGGSGGGGSGGGGSGGGGSGGGGSGGGGSLQIYIWAPLAGTCGVLLLSLVITGSGEGRGSLLTCGDVEENPGPMDWTWILFLVAAATRVHSNWVNVISDLKKIEDLIQSMHIDATLYTESDVHPSCKVTAMKCFLLELQVISLESGDASIHDTVENLIILANNSLSSNGNVTESGCKECEELEEKNIKEFLQSFVHIVQMFINTSSGGGGSGGGGSGGGGSGGGGSGGGSLQLLPSWAITLISVNGIFVICCLTYCFAPRCRERRRNERLRRESVRPV

SEQ ID NO: 35 - protein, 452 aa, synthetic construct
  REGION 1..452: note = synthetic
MDWTWILFLVAAATRVHSQGQDRHMIRMRQLIDIVDQLKNYVNDLVPEFLPAPEDVETNCEWSAFSCFQKAQLKSANTGNNERIINVSIKKLKRKPPSTNAGRRQKHRLTCPSCDSYEKKPPKEFLERFKSLLQKMIHQHLSSRTHGSEDSSGGGGSGGGGSGGGGSGGGGSGGGGSGGGGSGGGGSGGGGSGGGGSLQIYIWAPLAGTCGVLLLSLVITRAKRSGSGATNFSLLKQAGDVEENPGPMDWTWILFLVAAATRVHSNWVNVISDLKKIEDLIQSMHIDATLYTESDVHPSCKVTAMKCFLLELQVISLESGDASIHDTVENLIILANNSLSSNGNVTESGCKECEELEEKNIKEFLQSFVHIVQMFINTSSGGGGSGGGGSGGGGSGGGGSGGGSLQLLPSWAITLISVNGIFVICCLTYCFAPRCRERRRNERLRRESVRPV

SEQ ID NO: 36 - protein, 473 aa, synthetic construct
  REGION 1..473: note = synthetic
MDWTWILFLVAAATRVHSQGQDRHMIRMRQLIDIVDQLKNYVNDLVPEFLPAPEDVETNCEWSAFSCFQKAQLKSANTGNNERIINVSIKKLKRKPPSTNAGRRQKHRLTCPSCDSYEKKPPKEFLERFKSLLQKMIHQHLSSRTHGSEDSSGGGGSGGGGSGGGGSGGGGSGGGGSGGGGSGGGGSGGGGSGGGGSLQLLPSWAITLISVNGIFVICCLTYCFAPRCRERRRNERLRRESVRPVGSGQCTNYALLKLAGDVESNPGPMDWTWILFLVAAATRVHSNWVNVISDLKKIEDLIQSMHIDATLYTESDVHPSCKVTAMKCFLLELQVISLESGDASIHDTVENLIILANNSLSSNGNVTESGCKECEELEEKNIKEFLQSFVHIVQMFINTSSGGGGSGGGGSGGGGSGGGGSGGGSLQLLPSWAITLISVNGIFVICCLTYCFAPRCRERRRNERLRRESVRPV

SEQ ID NO: 37 - protein, 477 aa, synthetic construct
  REGION 1..477: note = synthetic
MDWTWILFLVAAATRVHSQGQDRHMIRMRQLIDIVDQLKNYVNDLVPEFLPAPEDVETNCEWSAFSCFQKAQLKSANTGNNERIINVSIKKLKRKPPSTNAGRRQKHRLTCPSCDSYEKKPPKEFLERFKSLLQKMIHQHLSSRTHGSEDSSGGGGSGGGGSGGGGSGGGGSGGGGSGGGGSGGGGSGGGGSGGGGSLQLLPSWAITLISVNGIFVICCLTYCFAPRCRERRRNERLRRESVRPVRAKRSGSGATNFSLLKQAGDVEENPGPMDWTWILFLVAAATRVHSNWVNVISDLKKIEDLIQSMHIDATLYTESDVHPSCKVTAMKCFLLELQVISLESGDASIHDTVENLIILANNSLSSNGNVTESGCKECEELEEKNIKEFLQSFVHIVQMFINTSSGGGGSGGGGSGGGGSGGGGSGGGSLQLLPSWAITLISVNGIFVICCLTYCFAPRCRERRRNERLRRESVRPV

SEQ ID NO: 38 - protein, 27 aa, Homo sapiens
NIKGSPWKGSLLLLLVSNLLLCQSVAP

SEQ ID NO: 39 - DNA, 1341 bp, synthetic construct
  misc_feature 1..1341: note = synthetic
  source 1..1341: mol_type = other DNA
atggattggacctggattctgttcctggtggccgctgccacaagagtgcatagccagggccaagaccggcacatgatccggatgagacagctgatcgacatcgtggaccagctgaagaactacgtgaacgacctggtgcctgagttcctgcctgctcctgaggacgtggaaacaaattgcgagtggtccgccttcagctgcttccagaaggcccagctgaaaagcgccaacaccggcaacaacgagcggatcatcaacgtgtccatcaagaagctgaagcggaagcctcctagcaccaatgccggaagaaggcagaagcacagactgacctgtcctagctgcgacagctacgagaagaagcctccaaaagagttcctggaacggttcaagagcctgctgcagaagatgatccaccagcacctgagcagcagaacccacggctctgaagattctagcggaggcggaggaagtggtggcggaggttctggtggcggtggatcaggcggtggcggatctggcggcggaggcagtggcggaggtggaagcggtggtggtggctctggcggaggcggtagcggcggaggcggatctcttcagatctatatttgggcccctctggccggaacatgtggcgtgttgctgctgtctctggttatcaccggcagcggcgccacaaatttcagcctgctgaaacaggccggcgacgtggaagagaatcctggacctatggactggacttggatactctttctggtcgctgccgccacacgggtgcactctaattgggtcaacgtgatcagcgacctgaagaagatcgaggacctgatccagagcatgcacatcgacgccacactgtacaccgagtccgatgtgcaccctagctgcaaagtgaccgccatgaagtgctttctgctggaactgcaagtgatcagcctggaaagcggcgacgccagcatccacgataccgtggaaaatctgatcatcctggccaacaacagcctgtccagcaacggcaatgtgaccgagagcggctgcaaagagtgcgaggaactggaagagaagaacatcaaagagtttctgcagagcttcgtccacatcgtgcagatgttcatcaacacctcatcaggcggcggtggtagtggaggcggaggctcaggcggcggaggttccggaggtggcggttccggcggaggatctcttcaattgctgcctagctgggccatcacactgatctccgtgaacggcatcttcgtgatctgctgcctgacctactgcttcgcccctagatgcagagagcggagaagaaacgagcggctgagaagagaaagcgtgcggcctgtg

SEQ ID NO: 40 - DNA, 1344 bp, synthetic construct
  misc_feature 1..1344: note = synthetic
  source 1..1344: mol_type = other DNA
atggattggacctggattctgttcctggtggccgctgccacaagagtgcatagccagggccaagaccggcacatgatccggatgagacagctgatcgacatcgtggaccagctgaagaactacgtgaacgacctggtgcctgagttcctgcctgctcctgaggacgtggaaacaaattgcgagtggtccgccttcagctgcttccagaaggcccagctgaaaagcgccaacaccggcaacaacgagcggatcatcaacgtgtccatcaagaagctgaagcggaagcctcctagcaccaatgccggaagaaggcagaagcacagactgacctgtcctagctgcgacagctacgagaagaagcctccaaaagagttcctggaacggttcaagagcctgctgcagaagatgatccaccagcacctgagcagcagaacccacggctctgaagattctagcggaggcggaggaagtggtggcggaggttctggtggcggtggatcaggcggtggcggatctggcggcggaggcagtggcggaggtggaagcggtggtggtggctctggcggaggcggtagcggcggaggcggatctcttcagatctatatttgggcccctctggccggaacatgtggcgtgttgctgctgtctctggttatcaccggctccggccagtgtaccaattacgccctgcttaaactggccggcgacgtggaatccaatcctggacctatggactggacttggatactctttctggtcgctgccgccacacgggtgcactctaattgggtcaacgtgatcagcgacctgaagaagatcgaggacctgatccagagcatgcacatcgacgccacactgtacaccgagtccgatgtgcaccctagctgcaaagtgaccgccatgaagtgctttctgctggaactgcaagtgatcagcctggaaagcggcgacgccagcatccacgataccgtggaaaatctgatcatcctggccaacaacagcctgtccagcaacggcaatgtgaccgagagcggctgcaaagagtgcgaggaactggaagagaagaacatcaaagagtttctgcagagcttcgtccacatcgtgcagatgttcatcaacacctcatcaggcggcggtggtagtggaggcggaggctcaggcggcggaggttccggaggtggcggttccggcggaggatctcttcaattgctgcctagctgggccatcacactgatctccgtgaacggcatcttcgtgatctgctgcctgacctactgcttcgcccctagatgcagagagcggagaagaaacgagcggctgagaagagaaagcgtgcggcctgtg

SEQ ID NO: 41 - DNA, 1338 bp, synthetic construct
  misc_feature 1..1338: note = synthetic
  source 1..1338: mol_type = other DNA
atggattggacctggattctgttcctggtggccgctgccacaagagtgcatagccagggccaagaccggcacatgatccggatgagacagctgatcgacatcgtggaccagctgaagaactacgtgaacgacctggtgcctgagttcctgcctgctcctgaggacgtggaaacaaattgcgagtggtccgccttcagctgcttccagaaggcccagctgaaaagcgccaacaccggcaacaacgagcggatcatcaacgtgtccatcaagaagctgaagcggaagcctcctagcaccaatgccggaagaaggcagaagcacagactgacctgtcctagctgcgacagctacgagaagaagcctccaaaagagttcctggaacggttcaagagcctgctgcagaagatgatccaccagcacctgagcagcagaacccacggctctgaagattctagcggaggcggaggaagtggtggcggaggttctggtggcggtggatcaggcggtggcggatctggcggcggaggcagtggcggaggtggaagcggtggtggtggctctggcggaggcggtagcggcggaggcggatctcttcagatctatatttgggcccctctggccggaacatgtggcgtgttgctgctgtctctggttatcaccggttctggcgaaggcagaggctctctgcttacttgtggcgacgtggaagagaatcctggacctatggactggacttggatactctttctggtcgctgccgccacacgggtgcactctaattgggtcaacgtgatcagcgacctgaagaagatcgaggacctgatccagagcatgcacatcgacgccacactgtacaccgagtccgatgtgcaccctagctgcaaagtgaccgccatgaagtgctttctgctggaactgcaagtgatcagcctggaaagcggcgacgccagcatccacgataccgtggaaaatctgatcatcctggccaacaacagcctgtccagcaacggcaatgtgaccgagagcggctgcaaagagtgcgaggaactggaagagaagaacatcaaagagtttctgcagagcttcgtccacatcgtgcagatgttcatcaacacctcatcaggcggcggtggtagtggaggcggaggctcaggcggcggaggttccggaggtggcggttccggcggaggatctcttcaattgctgcctagctgggccatcacactgatctccgtgaacggcatcttcgtgatctgctgcctgacctactgcttcgcccctagatgcagagagcggagaagaaacgagcggctgagaagagaaagcgtgcggcctgtg

SEQ ID NO: 42 - DNA, 1356 bp, synthetic construct
  misc_feature 1..1356: note = synthetic
  source 1..1356: mol_type = other DNA
atggattggacctggattctgttcctggtggccgctgccacaagagtgcatagccagggccaagaccggcacatgatccggatgagacagctgatcgacatcgtggaccagctgaagaactacgtgaacgacctggtgcctgagttcctgcctgctcctgaggacgtggaaacaaattgcgagtggtccgccttcagctgcttccagaaggcccagctgaaaagcgccaacaccggcaacaacgagcggatcatcaacgtgtccatcaagaagctgaagcggaagcctcctagcaccaatgccggaagaaggcagaagcacagactgacctgtcctagctgcgacagctacgagaagaagcctccaaaagagttcctggaacggttcaagagcctgctgcagaagatgatccaccagcacctgagcagcagaacccacggctctgaagattctagcggaggcggaggaagtggtggcggaggttctggtggcggtggatcaggcggtggcggatctggcggcggaggcagtggcggaggtggaagcggtggtggtggctctggcggaggcggtagcggcggaggcggatctcttcagatctatatttgggcccctctggccggaacatgtggcgtgttgctgctgtctctggttatcaccagggccaaaagaagcggcagcggcgccacaaatttcagcctgctgaaacaggccggcgacgtggaagagaatcctggacctatggactggacttggatactctttctggtcgctgccgccacacgggtgcactctaattgggtcaacgtgatcagcgacctgaagaagatcgaggacctgatccagagcatgcacatcgacgccacactgtacaccgagtccgatgtgcaccctagctgcaaagtgaccgccatgaagtgctttctgctggaactgcaagtgatcagcctggaaagcggcgacgccagcatccacgataccgtggaaaatctgatcatcctggccaacaacagcctgtccagcaacggcaatgtgaccgagagcggctgcaaagagtgcgaggaactggaagagaagaacatcaaagagtttctgcagagcttcgtccacatcgtgcagatgttcatcaacacctcatcaggcggcggtggtagtggaggcggaggctcaggcggcggaggttccggaggtggcggttccggcggaggatctcttcaattgctgcctagctgggccatcacactgatctccgtgaacggcatcttcgtgatctgctgcctgacctactgcttcgcccctagatgcagagagcggagaagaaacgagcggctgagaagagaaagcgtgcggcctgtg

SEQ ID NO: 43 - DNA, 1419 bp, synthetic construct
  misc_feature 1..1419: note = synthetic
  source 1..1419: mol_type = other DNA
atggattggacctggattctgttcctggtggccgctgccacaagagtgcatagccagggccaagaccggcacatgatccggatgagacagctgatcgacatcgtggaccagctgaagaactacgtgaacgacctggtgcctgagttcctgcctgctcctgaggacgtggaaacaaattgcgagtggtccgccttcagctgcttccagaaggcccagctgaaaagcgccaacaccggcaacaacgagcggatcatcaacgtgtccatcaagaagctgaagcggaagcctcctagcaccaatgccggaagaaggcagaagcacagactgacctgtcctagctgcgacagctacgagaagaagcctccaaaagagttcctggaacggttcaagagcctgctgcagaagatgatccaccagcacctgagcagcagaacccacggctctgaagattctagcggaggcggaggaagtggtggcggaggttctggtggcggtggatcaggcggtggcggatctggcggcggaggcagtggcggaggtggaagcggtggtggtggctctggcggaggcggtagcggcggaggcggatctcttcaattgctgcctagctgggccatcacactgatctccgtgaacggcatcttcgtgatctgctgcctgacctactgcttcgcccctagatgcagagagcggagaagaaacgagcggctgagaagagaatctgtgcggcctgttggctccggccagtgtacaaattatgccctgctgaagctggccggcgacgtggaatctaatcctggacctatggactggacttggatactctttctggtcgctgccgccacacgggtgcactctaattgggtcaacgtgatcagcgacctgaagaagatcgaggacctgatccagagcatgcacatcgacgccacactgtacaccgagtccgatgtgcaccctagctgcaaagtgaccgccatgaagtgctttctgctggaactgcaagtgatcagcctggaaagcggcgacgccagcatccacgataccgtggaaaatctgatcatcctggccaacaacagcctgtccagcaacggcaatgtgaccgagagcggctgcaaagagtgcgaggaactggaagaaaagaacatcaaagagtttctgcagagcttcgtccacatcgtgcagatgttcatcaacacctcatcaggtggcggtggaagcggaggtggcggtagtggcggcggaggctcaggcggcggaggttccggcggaggatctcttcagctcctgccatcttgggctatcaccctgattagtgtgaatgggatctttgtcatctgttgtctcacgtactgtttcgctccccggtgcagagagagaaggcgcaacgaaagactgcggagagaaagcgtcagacccgtg

SEQ ID NO: 44 - DNA, 1431 bp, synthetic construct
  misc_feature 1..1431: note = synthetic
  source 1..1431: mol_type = other DNA
atggattggacctggattctgttcctggtggccgctgccacaagagtgcatagccagggccaagaccggcacatgatccggatgagacagctgatcgacatcgtggaccagctgaagaactacgtgaacgacctggtgcctgagttcctgcctgctcctgaggacgtggaaacaaattgcgagtggtccgccttcagctgcttccagaaggcccagctgaaaagcgccaacaccggcaacaacgagcggatcatcaacgtgtccatcaagaagctgaagcggaagcctcctagcaccaatgccggaagaaggcagaagcacagactgacctgtcctagctgcgacagctacgagaagaagcctccaaaagagttcctggaacggttcaagagcctgctgcagaagatgatccaccagcacctgagcagcagaacccacggctctgaagattctagcggaggcggaggaagtggtggcggaggttctggtggcggtggatcaggcggtggcggatctggcggcggaggcagtggcggaggtggaagcggtggtggtggctctggcggaggcggtagcggcggaggcggatctcttcaattgctgcctagctgggccatcacactgatctccgtgaacggcatcttcgtgatctgctgcctgacctactgcttcgcccctagatgcagagagcggagaagaaacgagcggctgagaagagaatctgtgcggcctgttagagccaagagatctggaagcggcgccaccaactttagcctgctgaaacaggctggcgacgtggaagagaaccctggacctatggactggacttggatactctttctggtcgctgccgccacacgggtgcactctaattgggtcaacgtgatcagcgacctgaagaagatcgaggacctgatccagagcatgcacatcgacgccacactgtacaccgagtccgatgtgcaccctagctgcaaagtgaccgccatgaagtgctttctgctggaactgcaagtgatcagcctggaaagcggcgacgccagcatccacgataccgtggaaaatctgatcatcctggccaacaacagcctgtccagcaacggcaatgtgaccgagagcggctgcaaagagtgcgaggaactggaagaaaagaacatcaaagagtttctgcagagcttcgtccacatcgtgcagatgttcatcaacacctcatcaggtggcggtggaagcggaggtggcggtagtggcggcggaggctcaggcggcggaggttccggcggaggatctcttcagctcctgccatcttgggctatcaccctgattagtgtgaatgggatctttgtcatctgttgtctcacgtactgtttcgctccccggtgcagagagagaaggcgcaacgaaagactgcggagagaaagcgtcagacccgtg